European Patent Specification EP 3 464 575 B1, published May 6, 2026. Title: Transposase-random priming DNA sample preparation. Applicant: Agilent Technologies, Inc. The sequence listing filed with the application follows.

SEQUENCE LISTING (5 sequences)

SEQ ID NO: 1 - DNA, 19 bp, Artificial Sequence
  Synthetic oligonucleotide
ctgtctcttgatcacaagt

SEQ ID NO: 2 - DNA, 31 bp, Artificial Sequence
  Synthetic oligonucleotide
gctgacgtcgagacttgtgatcaagagacag

SEQ ID NO: 3 - DNA, 20 bp, Artificial Sequence
  Synthetic oligonucleotide
gctgacgtcgagacttgtga

SEQ ID NO: 4 - DNA, 33 bp, Artificial Sequence
  Synthetic oligonucleotide
  misc_feature (30)..(33): "n" is any nucleotide
agctgtgcgtagatgtgatcaagagacagnnnn

SEQ ID NO: 5 - DNA, 35 bp, Artificial Sequence
  Synthetic oligonucleotide
cggtggagctgtgcgtagatgtgatcaagagacag